European Patent Application EP 4 201 962 A1, published June 28, 2023. Title: Antibody Fragment Consisting of Cgamma1 and Cepsilon2-4 and Uses Thereof. Applicant: Ajou University Industry-Academic Cooperation Foundation. The sequence listing filed with the application follows.

SEQUENCE LISTING (7 sequences)

SEQ ID NO: 1 - protein, 436 aa, Artificial Sequence
  human Cgamma1 epsilon2-4
MASTKGPSVFPLAPSSKSTSGGTAALGCLVKDYFPEPVTVSWNSGALTSGVHTFPAVLQSSGLYSLSSVVTVPSSSLGTQTYICNVNHKPSNTKVDKKVEPKSCDKTHTCPVCSRDFTPPTVKILQSSCDGGGHFPPTIQLLCLVSGYTPGTINITWLEDGQVMDVDLSTASTTQEGELASTQSELTLSQKHWLSDRTYTCQVTYQGHTFEDSTKKCADSNPRGVSAYLSRPSPFDLFIRKSPTITCLVVDLAPSKGTVNLTWSRASGKPVNHSTRKEEKQRNGTLTVTSTLPVGTRDWIEGETYQCRVTHPHLPRALMRSTTKTSGPRAAPEVYAFATPEWPGSRDKRTLACLIQNFMPEDISVQWLHNEVQLPDARHSTTQPRKTKGSGFFVFSRLEVTRAEWEQKDEFICRAVHEAASPSQTVQRAVSVNPGK

SEQ ID NO: 2 - protein, 108 aa, Artificial Sequence
  human Ckappa
MRTVAAPSVFIFPPSDEQLKSGTASVVCLLNNFYPREAKVQWKVDNALQSGNSQESVTEQDSKDSTYSLSSTLTLSKADYEKHKVYACEVTHQGLSSPVTKSFNRGEC

SEQ ID NO: 3 - protein, 448 aa, Artificial Sequence
  6C407 IgE Heavy chain
EVQLQQSGAELVKPGASVKLSCTASGFNIKDTYIHWVKQRPEQGLEWIGRIDPANGNTKYDPKFQGKATITADTSSNTAYLQLSSLTSEDTAVYYCARGYGSRSAMDYWGQGTSVTVSASTKGPSVFPLAPSSKSTSGGTAALGCLVKDYFPEPVTVSWNSGALTSGVHTFPAVLQSSGLYSLSSVVTVPSSSLGTQTYICNVNHKPSNTKVDKKVEPKSCDKTHTCPPCPAPELLGGPSVFLFPPKPKDTLMISRTPEVTCVVVDVSHEDPEVKFNWYVDGVEVHNAKTKPREEQYNSTYRVVSVLTVLHQDWLNGKEYKCKVSNKALPAPIEKTISKAKGQPREPQVYTLPPSRDELTKNQVSLTCLVKGFYPSDIAVEWESNGQPENNYKTTPPVLDSDGSFFLYSKLTVDKSRWQQGNVFSCSVMHEALHNHYTQKSLSLSPGK

SEQ ID NO: 4 - protein, 220 aa, Artificial Sequence
  6C407 IgE Light chain
DIVLTQSPASLAVSLGQRATISCRASKSVSTSGYSYMLWYQQKPGQPPKLLIYLASNLESGVPARFSGSGSGTDFTLNIHPVEEEDAATYYCQHSRELPWTFGGGTKLEIKRARTVAAPSVFIFPPSDEQLKSGTASVVCLLNNFYPREAKVQWKVDNALQSGNSQESVTEQDSKDSTYSLSSTLTLSKADYEKHKVYACEVTHQGLSSPVTKSFNRGEC

SEQ ID NO: 5 - protein, 429 aa, Artificial Sequence
  Human Cepsilon
MASTQSPSVFPLTRCCKNIPSNATSVTLGCLATGYFPEPVMVTWDTGSLNGTTMTLPATTLTLSGHYATISLLTVSGAWAKQMFTCRVAHTPSSTDWVDNKTFSVCSRDFTPPTVKILQSSCDGGGHFPPTIQLLCLVSGYTPGTINITWLEDGQVMDVDLSTASTTQEGELASTQSELTLSQKHWLSDRTYTCQVTYQGHTFEDSTKKCADSNPRGVSAYLSRPSPFDLFIRKSPTITCLVVDLAPSKGTVNLTWSRASGKPVNHSTRKEEKQRNGTLTVTSTLPVGTRDWIEGETYQCRVTHPHLPRALMRSTTKTSGPRAAPEVYAFATPEWPGSRDKRTLACLIQNFMPEDISVQWLHNEVQLPDARHSTTQPRKTKGSGFFVFSRLEVTRAEWEQKDEFICRAVHEAASPSQTVQRAVSVNPGK

SEQ ID NO: 6 - protein, 108 aa, Artificial Sequence; identical to SEQ ID NO: 2
  Human Ckappa

SEQ ID NO: 7 - protein, 552 aa, Artificial Sequence
  IgCwepsilonLkappa
MRTVAAPSVFIFPPSDEQLKSGTASVVCLLNNFYPREAKVQWKVDNALQSGNSQESVTEQDSKDSTYSLSSTLTLSKADYEKHKVYACEVTHQGLSSPVTKSFNRGECGGGGSGGGGSGGGGSMASTQSPSVFPLTRCCKNIPSNATSVTLGCLATGYFPEPVMVTWDTGSLNGTTMTLPATTLTLSGHYATISLLTVSGAWAKQMFTCRVAHTPSSTDWVDNKTFSVCSRDFTPPTVKILQSSCDGGGHFPPTIQLLCLVSGYTPGTINITWLEDGQVMDVDLSTASTTQEGELASTQSELTLSQKHWLSDRTYTCQVTYQGHTFEDSTKKCADSNPRGVSAYLSRPSPFDLFIRKSPTITCLVVDLAPSKGTVNLTWSRASGKPVNHSTRKEEKQRNGTLTVTSTLPVGTRDWIEGETYQCRVTHPHLPRALMRSTTKTSGPRAAPEVYAFATPEWPGSRDKRTLACLIQNFMPEDISVQWLHNEVQLPDARHSTTQPRKTKGSGFFVFSRLEVTRAEWEQKDEFICRAVHEAASPSQTVQRAVSVNPGK